European Patent Specification EP 3 307 774 B1, published April 30, 2025. Title: Monoclonal antibodies specific for serogroup X of N. meningitidis and uses thereof in diagnosis. Applicant: Institut Pasteur. The sequence listing filed with the application follows.

SEQUENCE LISTING (13 sequences)

SEQ ID NO: 1 - protein, 7 aa, Mus musculus
GFSLTSY

SEQ ID NO: 2 - protein, 6 aa, Mus musculus
IWAGGS

SEQ ID NO: 3 - protein, 11 aa, Mus musculus
ARALLRGAMDY

SEQ ID NO: 4 - protein, 11 aa, Mus musculus
QSLVHSNGNTY

SEQ ID NO: 5 - protein, 3 aa, Mus musculus
KVS

SEQ ID NO: 6 - protein, 9 aa, Mus musculus
SQSTHVPPT

SEQ ID NO: 7 - protein, 120 aa, Mus musculus
IGLVAPSQSMYITCTVSGFSLTSYGVHWVRQPPGKGLEWLGVIWAGGSTNYNSALMSRLSISKDNSKSQVFLKMNSLQTDDTAMYYCARALLRGAMDYWGQGTSVTVSSESQSFPNVFPL

SEQ ID NO: 8 - protein, 120 aa, Mus musculus
IGLVAPSQSLSITCTVSGFSLTSYGVHWVRQPPGKGLEWLGVIWAGGSTNYNSALMSRLSISKDNSKSQVFLKMNSLQTDDTAMYYCARALLRGAMDYWGQGTSVTVSSESQSFPNVFPL

SEQ ID NO: 9 - protein, 120 aa, Mus musculus
LSLPVSLGDQASISCRSSQSLVHSNGNTYLHWYLQKPGQSPKLLIYKVSNRFSGVPDRFSGSGSGTDFTLKISRVEAEDLGVYFCSQSTHVPPTFGGGTKLEIKRADAAPTVSIFPPSSE

SEQ ID NO: 10 - DNA, 31 bp, artificial
  primer for IgM Heavy chain
atgcagactagtgtttttgcctccgtagtgg

SEQ ID NO: 11 - DNA, 33 bp, artificial
  primer for IgM Heavy chain
cctaggggaggtgcagcttgaggagtcaggacc

SEQ ID NO: 12 - DNA, 28 bp, artificial
  primer for IgM light chain
ttctagactaacactcattcctgttgaa

SEQ ID NO: 13 - DNA, 31 bp, artificial
  primer for IgM Light chain
aagatctgagctcgtgatgacccagactcca